European Patent Specification EP 3 247 721 B1, published May 7, 2025. Title: IgG Bispecific Antibodies and Processes for Preparation. Applicant: Eli Lilly and Company. The sequence listing filed with the application follows.

SEQUENCE LISTING (69 sequences)

SEQ ID NO: 1 - protein, 449 aa, Artificial Sequence
  Synthetic Construct
EVQLVESGGGLVQPGGSLRLSCAASGYTFTSYWLHWVRQAPGKGLEWVGMIDPSNSDTRFNPNFKDRFTISADTSKNTAYLQMNSLRAEDTAVYYCATYRSYVTPLDYWGQGTLVTVSSASTKGPSVFPLAPSSKSTSGGTAALGCLVKDYFPEPVTVSWNSGALTSGVHTFPAVLQSSGLYSLSSVVTVPSSSLGTQTYICNVNHKPSNTKVDKRVEPKSCDKTHTCPPCPAPELLGGPSVFLFPPKPKDTLMISRTPEVTCVVVDVSHEDPEVKFNWYVDGVEVHNAKTKPREEQYNSTYRVVSVLTVLHQDWLNGKEYKCKVSNKALPAPIEKTISKAKGQPREPQVYTLPPSREEMTKNQVSLTCLVKGFYPSDIAVEWESNGQPENNYKTTPPVLDSDGSFFLYSKLTVDKSRWQQGNVFSCSVMHEALHNHYTQKSLSLSPGK

SEQ ID NO: 2 - protein, 241 aa, Artificial Sequence
  Synthetic Construct
YPYDVPDYASGSGSDKTHTCPPCPAPELLGGPSVFLFPPKPKDTLMISRTPEVTCVVVDVSHEDPEVKFNWYVDGVEVHNAKTKPREEQYNSTYRVVSVLTVLHQDWLNGKEYKCKVSNKALPAPIEKTISKAKGQPREPQVYTLPPSREEMTKNQVSLTCLVKGFYPSDIAVEWESNGQPENNYKTTPPVLDSDGSFFLYSKLTVDKSRWQQGNVFSCSVMHEALHNHYTQKSLSLSPGK

SEQ ID NO: 3 - protein, 220 aa, Artificial Sequence
  Synthetic Construct
DIQMTQSPSSLSASVGDRVTITCKSSQSLLYTSSQKNYLAWYQQKPGKAPKLLIYWASTRESGVPSRFSGSGSGTDFTLTISSLQPEDFATYYCQQYYAYPWTFGQGTKVEIKRTVAAPSVFIFPPSDEQLKSGTASVVCLLNNFYPREAKVQWKVDNALQSGNSQESVTEQDSKDSTYSLSSTLTLSKADYEKHKVYACEVTHQGLSSPVTKSFNRGEC

SEQ ID NO: 4 - protein, 449 aa, Artificial Sequence
  Synthetic Construct
EQKLISEEDLSGSEERKVCNGIGIGEFKDSLSINATNIKHFKNCTSISGDLHILPVAFRGDSFTHTPPLDPQELDILKTVKEITGFLLIQAWPENRTDLHAFENLEIIRGRTKQHGQFSLAVVSLNITSLGLRSLKEISDGDVIISGNKNLCYANTINWKKLFGTSGQKTKIISNRGENSCKATGQVCHALCSPEGCWGPEPRDCVSCRNVSRGRECVDKGSDKTHTCPPCPAPELLGGPSVFLFPPKPKDTLMISRTPEVTCVVVDVSHEDPEVKFNWYVDGVEVHNAKTKPREEQYNSTYRVVSVLTVLHQDWLNGKEYKCKVSNKALPAPIEKTISKAKGQPREPQVYTLPPSREEMTKNQVSLTCLVKGFYPSDIAVEWESNGQPENNYKTTPPVLDSDGSFFLYSKLTVDKSRWQQGNVFSCSVMHEALHNHYTQKSLSLSPGK

SEQ ID NO: 5 - protein, 345 aa, Artificial Sequence
  Synthetic Construct
EQKLISEEDLSGSQTNTILDVQIRPPSPVRLLHGQTLVLNCTATTELNTRVQMSWNYPGKATKRASIRQRIDRSHSHNNVFHSVLKINNVESRDKGLYTCRVKSGSSFQSFNTSVHGSDKTHTCPPCPAPELLGGPSVFLFPPKPKDTLMISRTPEVTCVVVDVSHEDPEVKFNWYVDGVEVHNAKTKPREEQYNSTYRVVSVLTVLHQDWLNGKEYKCKVSNKALPAPIEKTISKAKGQPREPQVYTLPPSREEMTKNQVSLTCLVKGFYPSDIAVEWESNGQPENNYKTTPPVLDSDGSFFLYSKLTVDKSRWQQGNVFSCSVMHEALHNHYTQKSLSLSPGK

SEQ ID NO: 6 - protein, 227 aa, Artificial Sequence
  Synthetic Construct
DKTHTCPPCPAPELLGGPSVFLFPPKPKDTLMISRTPEVTCVVVDVSHEDPEVKFNWYVDGVEVHNAKTKPREEQYNSTYRVVSVLTVLHQDWLNGKEYKCKVSNKALPAPIEKTISKAKGQPREPQVYTLPPSREEMTKNQVSLTCLVKGFYPSDIAVEWESNGQPENNYKTTPPVLDSDGSFFLYSKLTVDKSRWQQGNVFSCSVMHEALHNHYTQKSLSLSPGK

SEQ ID NO: 7 - protein, 217 aa, Artificial Sequence
  Synthetic Construct
APELLGGPSVFLFPPKPKDTLMISRTPEVTCVVVDVSHEDPEVKFNWYVDGVEVHNAKTKPREEQYNSTYRVVSVLTVLHQDWLNGKEYKCKVSNKALPAPIEKTISKAKGQPREPQVYTLPPSREEMTKNQVSLTCLVKGFYPSDIAVEWESNGQPENNYKTTPPVLDSDGSFFLASKLTVDKSRWQQGNVFSCSVMHEALHNHYTQKSLSLSPGK

SEQ ID NO: 8 - protein, 217 aa, Artificial Sequence
  Synthetic Construct
APELLGGPSVFLFPPKPKDTLMISRTPEVTCVVVDVSHEDPEVKFNWYVDGVEVHNAKTKPREEQYNSTYRVVSVLTVLHQDWLNGKEYKCKVSNKALPAPIEKTISKAKGQPREPQVYTLPPSREEMTKNQVSLMCLVKGFYPSDIAVEWESNGQPENNYKTTPPVLDSDGSFFLYSVLTVDKSRWQQGNVFSCSVMHEALHNHYTQKSLSLSPGK

SEQ ID NO: 9 - protein, 449 aa, Artificial Sequence
  Synthetic Construct
EVQLVESGGGLVQPGGSLRLSCAASGFTFTDYTMDWVRKAPGKGLEWVADVNPNSGGSIYNQEFKGRFTLSVDRSKNTLYLQMNSLRAEDTAVYYCARNLGPSFYFDYWGQGTLVTVSSASTKGPSVFPLAPSSKSTSGGTAALGCLVKDYFPEPVTVSWNSGALTSGVATGPAVLQSSGLYSLSSVVTVPSSSLGTQTYICNVNHKPSNTKVDKKVEPKSCDKTHTCPPCPAPELLGGPSVFLFPPKPKDTLMISRTPEVTCVVVDVSHEDPEVKFNWYVDGVEVHNAKTKPREEQYQSTYRVVSVLTVLHQDWLNGKEYKCKVSNKALPAPIEKTISKAKGQPREPQVYTLPPSREEMTKNQVSLTCLVKGFYPSDIAVEWESNGQPENNYKTTPPVLDSDGSFFLYSKLTVDKSRWQQGNVFSCSVMHEALHNHYTQKSLSLSPGK

SEQ ID NO: 10 - protein, 449 aa, Artificial Sequence
  Synthetic Construct
EVQLVESGGGLVQPGGSLRLSCAASGFTFTDYTMDWVRKAPGKGLEWVADVNPNSGGSIYNQEFKGRFTLSVDRSKNTLYLQMNSLRAEDTAVYYCARNLGPSFYFDYWGQGTLVTVSSASTKGPSVFPLAPSSKSTSGGTAALGCLVKDYFPEPVTVSWNSGALTSGVATGPAVLQSSGLYSLSSVVTVPSSSLGTQTYICNVNHKPSNTKVDKKVEPKSCDKTHTCPPCPAPELLGGPSVFLFPPKPKDTLMISRTPEVTCVVVDVSHEDPEVKFNWYVDGVEVHNAKTKPREEQYQSTYRVVSVLTVLHQDWLNGKEYKCKVSNKALPAPIEKTISKAKGQPREPQVYTLPPSREEMTKNQVSLTCLVKGFYPSDIAVEWESNGQPENNYKTTPPVLMSDGSFFLASKLTVDKSRWQQGNVFSCSVMHEALHNHYTQKSLSLSPGK

SEQ ID NO: 11 - protein, 449 aa, Artificial Sequence
  Synthetic Construct
EVQLVESGGGLVQPGGSLRLSCAASGFTFTDYTMDWVRKAPGKGLEWVADVNPNSGGSIYNQEFKGRFTLSVDRSKNTLYLQMNSLRAEDTAVYYCARNLGPSFYFDYWGQGTLVTVSSASTKGPSVFPLAPSSKSTSGGTAALGCLVKDYFPEPVTVSWNSGALTSGVATGPAVLQSSGLYSLSSVVTVPSSSLGTQTYICNVNHKPSNTKVDKKVEPKSCDKTHTCPPCPAPELLGGPSVFLFPPKPKDTLMISRTPEVTCVVVDVSHEDPEVKFNWYVDGVEVHNAKTKPREEQYQSTYRVVSVLTVLHQDWLNGKEYKCKVSNKALPAPIEKTISKAKGQPREPQVYTLPPSREEMTDNQVSLTCLVKGFYPSDIAVEWESNGQPENNYKTTPPVLMSDGSFFLASKLTVDKSRWQQGNVFSCSVMHEALHNHYTQKSLSLSPGK

SEQ ID NO: 12 - protein, 449 aa, Artificial Sequence
  Synthetic Construct
EVQLVESGGGLVQPGGSLRLSCAASGFTFTDYTMDWVRKAPGKGLEWVADVNPNSGGSIYNQEFKGRFTLSVDRSKNTLYLQMNSLRAEDTAVYYCARNLGPSFYFDYWGQGTLVTVSSASTKGPSVFPLAPSSKSTSGGTAALGCLVKDYFPEPVTVSWNSGALTSGVATGPAVLQSSGLYSLSSVVTVPSSSLGTQTYICNVNHKPSNTKVDKKVEPKSCDKTHTCPPCPAPELLGGPSVFLFPPKPKDTLMISRTPEVTCVVVDVSHEDPEVKFNWYVDGVEVHNAKTKPREEQYQSTYRVVSVLTVLHQDWLNGKEYKCKVSNKALPAPIEKTISKAKGQPREPQVSTLPPSREEMTKNQVSLVCLVYGFYPSDIAVEWESNGQPENNYKTTPPVLDSDGSFFLYSVLTVDKSRWQQGNVFSCSVMHEALHNHYTQKSLSLSPGK

SEQ ID NO: 13 - protein, 449 aa, Artificial Sequence
  Synthetic Construct
EVQLVESGGGLVQPGGSLRLSCAASGFTFTDYTMDWVRKAPGKGLEWVADVNPNSGGSIYNQEFKGRFTLSVDRSKNTLYLQMNSLRAEDTAVYYCARNLGPSFYFDYWGQGTLVTVSSASTKGPSVFPLAPSSKSTSGGTAALGCLVKDYFPEPVTVSWNSGALTSGVATGPAVLQSSGLYSLSSVVTVPSSSLGTQTYICNVNHKPSNTKVDKKVEPKSCDKTHTCPPCPAPELLGGPSVFLFPPKPKDTLMISRTPEVTCVVVDVSHEDPEVKFNWYVDGVEVHNAKTKPREEQYQSTYRVVSVLTVLHQDWLNGKEYKCKVSNKALPAPIEKTISKAKGQPREPQVSTLPPSREEMTKNQVSLMCLVYGFYPSDIAVEWESNGQPENNYKTTPPVLDSDGSFFLYSVLTVDKSRWQQGNVFSCSVMHEALHNHYTQKSLSLSPGK

SEQ ID NO: 14 - protein, 212 aa, Artificial Sequence
  Synthetic Construct
RIQMTQSPSSLSASVGDRVTITCKASQDVSIGVAWYQDKPGKAPKLLIYSASYRYTGVPSRFSGSGSGTDFTLTISSLQPEDFATYYCQQYYIYPYTFGQGTKVEIKGQPKAAPSVTLFPPSSEELQANKATLVCYISDFYPGAVTVAWKADSSPVKAGVETTTPSKQSNNKYAAWSYLSLTPEQWKSHRSYSCQVTHEGSTVEKTVAPTEC

SEQ ID NO: 15 - protein, 449 aa, Artificial Sequence
  Synthetic Construct
EVQLVESGGGLVQPGGSLRLSCAASGYTFTSYWLHWVRKAPGKGLEWVGMIDPSNSDTRFNPEFKDRFTISADTSKNTAYLQMNSLRAEDTAVYYCATYRSYVTPLDYWGQGTLVTVSSASTKGPSVFPLAPSSKSTSGGTAALGCLVKDYFPEPVTVSWNSGALTSGVATGPAVLQSSGLYSLSSVVTVPSSSLGTQTYICNVNHKPSNTKVDKKVEPKSCDKTHTCPPCPAPELLGGPSVFLFPPKPKDTLMISRTPEVTCVVVDVSHEDPEVKFNWYVDGVEVHNAKTKPREEQYQSTYRVVSVLTVLHQDWLNGKEYKCKVSNKALPAPIEKTISKAKGQPREPQVYTLPPSREEMTKNQVSLTCLVKGFYPSDIAVEWESNGQPENNYKTTPPVLDSDGSFFLYSKLTVDKSRWQQGNVFSCSVMHEALHNHYTQKSLSLSPGK

SEQ ID NO: 16 - protein, 449 aa, Artificial Sequence
  Synthetic Construct
EVQLVESGGGLVQPGGSLRLSCAASGYTFTSYWLHWVRKAPGKGLEWVGMIDPSNSDTRFNPEFKDRFTISADTSKNTAYLQMNSLRAEDTAVYYCATYRSYVTPLDYWGQGTLVTVSSASTKGPSVFPLAPSSKSTSGGTAALGCLVKDYFPEPVTVSWNSGALTSGVATGPAVLQSSGLYSLSSVVTVPSSSLGTQTYICNVNHKPSNTKVDKKVEPKSCDKTHTCPPCPAPELLGGPSVFLFPPKPKDTLMISRTPEVTCVVVDVSHEDPEVKFNWYVDGVEVHNAKTKPREEQYQSTYRVVSVLTVLHQDWLNGKEYKCKVSNKALPAPIEKTISKAKGQPREPQVYTLPPSREEMTKNQVSLVCLVKGFYPSDIAVEWESNGQPENNYKTTPPVLDSDGSFFLYSVLTVDKSRWQQGNVFSCSVMHEALHNHYTQKSLSLSPGK

SEQ ID NO: 17 - protein, 449 aa, Artificial Sequence
  Synthetic Construct
EVQLVESGGGLVQPGGSLRLSCAASGYTFTSYWLHWVRKAPGKGLEWVGMIDPSNSDTRFNPEFKDRFTISADTSKNTAYLQMNSLRAEDTAVYYCATYRSYVTPLDYWGQGTLVTVSSASTKGPSVFPLAPSSKSTSGGTAALGCLVKDYFPEPVTVSWNSGALTSGVATGPAVLQSSGLYSLSSVVTVPSSSLGTQTYICNVNHKPSNTKVDKKVEPKSCDKTHTCPPCPAPELLGGPSVFLFPPKPKDTLMISRTPEVTCVVVDVSHEDPEVKFNWYVDGVEVHNAKTKPREEQYQSTYRVVSVLTVLHQDWLNGKEYKCKVSNKALPAPIEKTISKAKGQPRRPRVYTLPPSREEMTKNQVSLVCLVKGFYPSDIAVEWESNGQPENNYKTTPPVLDSDGSFFLYSVLTVDKSRWQQGNVFSCSVMHEALHNHYTQKSLSLSPGK

SEQ ID NO: 18 - protein, 449 aa, Artificial Sequence
  Synthetic Construct
EVQLVESGGGLVQPGGSLRLSCAASGYTFTSYWLHWVRKAPGKGLEWVGMIDPSNSDTRFNPEFKDRFTISADTSKNTAYLQMNSLRAEDTAVYYCATYRSYVTPLDYWGQGTLVTVSSASTKGPSVFPLAPSSKSTSGGTAALGCLVKDYFPEPVTVSWNSGALTSGVATGPAVLQSSGLYSLSSVVTVPSSSLGTQTYICNVNHKPSNTKVDKKVEPKSCDKTHTCPPCPAPELLGGPSVFLFPPKPKDTLMISRTPEVTCVVVDVSHEDPEVKFNWYVDGVEVHNAKTKPREEQYQSTYRVVSVLTVLHQDWLNGKEYKCKVSNKALPAPIEKTISKAKGQPREPQVSTLPPSREEMTKNQVSLVCLVYGFYPSDIAVEWESNGQPENNYKTTPPVLDSDGSFFLYSVLTVDKSRWQQGNVFSCSVMHEALHNHYTQKSLSLSPGK

SEQ ID NO: 19 - protein, 449 aa, Artificial Sequence
  Synthetic Construct
EVQLVESGGGLVQPGGSLRLSCAASGYTFTSYWLHWVRKAPGKGLEWVGMIDPSNSDTRFNPEFKDRFTISADTSKNTAYLQMNSLRAEDTAVYYCATYRSYVTPLDYWGQGTLVTVSSASTKGPSVFPLAPSSKSTSGGTAALGCLVKDYFPEPVTVSWNSGALTSGVATGPAVLQSSGLYSLSSVVTVPSSSLGTQTYICNVNHKPSNTKVDKKVEPKSCDKTHTCPPCPAPELLGGPSVFLFPPKPKDTLMISRTPEVTCVVVDVSHEDPEVKFNWYVDGVEVHNAKTKPREEQYQSTYRVVSVLTVLHQDWLNGKEYKCKVSNKALPAPIEKTISKAKGQPREPQVSTLPPSREEMTKNQVSLMCLVYGFYPSDIAVEWESNGQPENNYKTTPPVLDSDGSFFLYSVLTVDKSRWQQGNVFSCSVMHEALHNHYTQKSLSLSPGK

SEQ ID NO: 20 - protein, 218 aa, Artificial Sequence
  Synthetic Construct
RIQMTQSPSSLSASVGDRVTITCKSSQSLLYTSSQKNYLAWYQDKPGKAPKLLIYWASTRESGVPSRFSGSGSGTDFTLTISSLQPEDFATYYCQQYYAYPWTFGQGTKVEIKGQPKAAPSVTLFPPSSEELQANKATLVCYISDFYPGAVTVAWKADSSPVKAGVETTTPSKQSNNKYAAWSYLSLTPEQWKSHRSYSCQVTHEGSTVEKTVAPTEC

SEQ ID NO: 21 - protein, 446 aa, Artificial Sequence
  Synthetic Construct
QVQLVQSGAEVKKPGSSVKVSCKASGYTFTTYYLHWVRYAPGQGLEWMGWIYPGNVHAQYNEKFKGRVTITADKSTSTAYMELSSLRSEDTAVYYCARSWEGFPYWGRGTTVTVSSASTKGPSVFPLAPCSKSTSGGTAALGCLVKDYFPEPVTVSWNSGALTSGVHTFPAVLQSSGLYSLSSVVTVPSSSLGTQTYICNVNHKPSNTKVDKKVEPDSGDKTHTCPPCPAPELLGGPSVFLFPPKPKDTLMISRTPEVTCVVVDVSHEDPEVKFNWYVDGVEVHNAKTKPREEQYNSTYRVVSVLTVLHQDWLNGKEYKCKVSNKALPAPIEKTISKAKGQPREPQVYTLPPSREEMTKNQVSLTCLVKGFYPSDIAVEWESNGQPENNYKTTPPVLDSDGSFFLYSKLTVDKSRWQQGNVFSCSVMHEALHNHYTQKSLSLSPGK

SEQ ID NO: 22 - protein, 446 aa, Artificial Sequence
  Synthetic Construct
QVQLVQSGAEVKKPGSSVKVSCKASGYTFTTYYLHWVRYAPGQGLEWMGWIYPGNVHAQYNEKFKGRVTITADKSTSTAYMELSSLRSEDTAVYYCARSWEGFPYWGRGTTVTVSSASTKGPSVFPLAPCSKSTSGGTAALGCLVKDYFPEPVTVSWNSGALTSGVHTFPAVLQSSGLYSLSSVVTVPSSSLGTQTYICNVNHKPSNTKVDKKVEPDSGDKTHTCPPCPAPELLGGPSVFLFPPKPKDTLMISRTPEVTCVVVDVSHEDPEVKFNWYVDGVEVHNAKTKPREEQYNSTYRVVSVLTVLHQDWLNGKEYKCKVSNKALPAPIEKTISKAKGQPREPQVYTLPPSREEMTKNQVSLVCLVKGFYPSDIAVEWESNGQPENNYKTTPPVLDSDGSFFLYSVLTVDKSRWQQGNVFSCSVMHEALHNHYTQKSLSLSPGK

SEQ ID NO: 23 - protein, 446 aa, Artificial Sequence
  Synthetic Construct
QVQLVQSGAEVKKPGSSVKVSCKASGYTFTTYYLHWVRYAPGQGLEWMGWIYPGNVHAQYNEKFKGRVTITADKSTSTAYMELSSLRSEDTAVYYCARSWEGFPYWGRGTTVTVSSASTKGPSVFPLAPCSKSTSGGTAALGCLVKDYFPEPVTVSWNSGALTSGVHTFPAVLQSSGLYSLSSVVTVPSSSLGTQTYICNVNHKPSNTKVDKKVEPDSGDKTHTCPPCPAPELLGGPSVFLFPPKPKDTLMISRTPEVTCVVVDVSHEDPEVKFNWYVDGVEVHNAKTKPREEQYNSTYRVVSVLTVLHQDWLNGKEYKCKVSNKALPAPIEKTISKAKGQPRRPRVYTLPPSREEMTKNQVSLVCLVKGFYPSDIAVEWESNGQPENNYKTTPPVLDSDGSFFLYSVLTVDKSRWQQGNVFSCSVMHEALHNHYTQKSLSLSPGK

SEQ ID NO: 24 - protein, 446 aa, Artificial Sequence
  Synthetic Construct
QVQLVQSGAEVKKPGSSVKVSCKASGYTFTTYYLHWVRYAPGQGLEWMGWIYPGNVHAQYNEKFKGRVTITADKSTSTAYMELSSLRSEDTAVYYCARSWEGFPYWGRGTTVTVSSASTKGPSVFPLAPCSKSTSGGTAALGCLVKDYFPEPVTVSWNSGALTSGVHTFPAVLQSSGLYSLSSVVTVPSSSLGTQTYICNVNHKPSNTKVDKKVEPDSGDKTHTCPPCPAPELLGGPSVFLFPPKPKDTLMISRTPEVTCVVVDVSHEDPEVKFNWYVDGVEVHNAKTKPREEQYNSTYRVVSVLTVLHQDWLNGKEYKCKVSNKALPAPIEKTISKAKGQPREPQVYTLPPSREDMTKNQVQLTCLVKGFYPSDIAVEWESNGQPENNYKTTPPVLDSDGSFFLASKLTVDKSRWQQGNVFSCSVMHEALHNHYTQKSLSLSPGK

SEQ ID NO: 25 - protein, 446 aa, Artificial Sequence
  Synthetic Construct
QVQLVQSGAEVKKPGSSVKVSCKASGYTFTTYYLHWVRYAPGQGLEWMGWIYPGNVHAQYNEKFKGRVTITADKSTSTAYMELSSLRSEDTAVYYCARSWEGFPYWGRGTTVTVSSASTKGPSVFPLAPCSKSTSGGTAALGCLVKDYFPEPVTVSWNSGALTSGVHTFPAVLQSSGLYSLSSVVTVPSSSLGTQTYICNVNHKPSNTKVDKKVEPDSGDKTHTCPPCPAPELLGGPSVFLFPPKPKDTLMISRTPEVTCVVVDVSHEDPEVKFNWYVDGVEVHNAKTKPREEQYNSTYRVVSVLTVLHQDWLNGKEYKCKVSNKALPAPIEKTISKAKGQPREPQVYTLPPSRGDMTKNQVQLTCLVKGFYPSDIAVEWESNGQPENNYKTTPPVLDSDGSFFLASKLTVDKSRWQQGNVFSCSVMHEALHNHYTQKSLSLSPGK

SEQ ID NO: 26 - protein, 446 aa, Artificial Sequence
  Synthetic Construct
QVQLVQSGAEVKKPGSSVKVSCKASGYTFTTYYLHWVRYAPGQGLEWMGWIYPGNVHAQYNEKFKGRVTITADKSTSTAYMELSSLRSEDTAVYYCARSWEGFPYWGRGTTVTVSSASTKGPSVFPLAPCSKSTSGGTAALGCLVKDYFPEPVTVSWNSGALTSGVHTFPAVLQSSGLYSLSSVVTVPSSSLGTQTYICNVNHKPSNTKVDKKVEPDSGDKTHTCPPCPAPELLGGPSVFLFPPKPKDTLMISRTPEVTCVVVDVSHEDPEVKFNWYVDGVEVHNAKTKPREEQYNSTYRVVSVLTVLHQDWLNGKEYKCKVSNKALPAPIEKTISKAKGQPREPQVYTLPPSREDMTKNQVRLTCLVKGFYPSDIAVEWESNGQPENNYKTTPPVLDSDGSFFLASKLTVDKSRWQQGNVFSCSVMHEALHNHYTQKSLSLSPGK

SEQ ID NO: 27 - protein, 214 aa, Artificial Sequence
  Synthetic Construct
DIQMTQSPSSLSASVGDRVTITCKASQNVGINVAWYQRKPGDAPKSLISSASYRYSGVPSRFSGSGSGTDFTLTISSLQPEDFATYFCQQYDTYPFTFGQGTKVEIKRTVAAPSVFIFPPSKEQLKSGTASVVCLLNNFYPREAKVQWKVDNALQSGNSQESVTEQDSKDSTYSLSSTLTLSKADYEKHKVYACEVTHQGLSSPVTKSFNRGEC

SEQ ID NO: 28 - protein, 451 aa, Artificial Sequence
  Synthetic Construct
QVQLVQSGAEVKKPGASVKVSCKASGYTFTSHWMHWVRYAPGQGLEWIGEFNPSNGRTNYNEKFKSKATMTVDTSTNTAYMELSSLRSEDTAVYYCASRDYDYDGRYFDYWGRGTLVTVSSASTKGPSVFPLAPCSKSTSGGTAALGCLVKDYFPEPVTVSWNSGALTSGVHTFPAVLQSSGLYSLSSVVTVPSSSLGTQTYICNVNHKPSNTKVDKKVEPDSGDKTHTCPPCPAPELLGGPSVFLFPPKPKDTLMISRTPEVTCVVVDVSHEDPEVKFNWYVDGVEVHNAKTKPREEQYNSTYRVVSVLTVLHQDWLNGKEYKCKVSNKALPAPIEKTISKAKGQPREPQVYTLPPSREEMTKNQVSLTCLVKGFYPSDIAVEWESNGQPENNYKTTPPVLDSDGSFFLYSKLTVDKSRWQQGNVFSCSVMHEALHNHYTQKSLSLSPGK

SEQ ID NO: 29 - protein, 451 aa, Artificial Sequence
  Synthetic Construct
QVQLVQSGAEVKKPGASVKVSCKASGYTFTSHWMHWVRYAPGQGLEWIGEFNPSNGRTNYNEKFKSKATMTVDTSTNTAYMELSSLRSEDTAVYYCASRDYDYDGRYFDYWGRGTLVTVSSASTKGPSVFPLAPCSKSTSGGTAALGCLVKDYFPEPVTVSWNSGALTSGVHTFPAVLQSSGLYSLSSVVTVPSSSLGTQTYICNVNHKPSNTKVDKKVEPDSGDKTHTCPPCPAPELLGGPSVFLFPPKPKDTLMISRTPEVTCVVVDVSHEDPEVKFNWYVDGVEVHNAKTKPREEQYNSTYRVVSVLTVLHQDWLNGKEYKCKVSNKALPAPIEKTISKAKGQPREPQVYTLPPSREEMTKNQVSLTCLVKGFYPSDIAVEWESNGQPENNYKTTPPVLMSDGSFFLASKLTVDKSRWQQGNVFSCSVMHEALHNHYTQKSLSLSPGK

SEQ ID NO: 30 - protein, 451 aa, Artificial Sequence
  Synthetic Construct
QVQLVQSGAEVKKPGASVKVSCKASGYTFTSHWMHWVRYAPGQGLEWIGEFNPSNGRTNYNEKFKSKATMTVDTSTNTAYMELSSLRSEDTAVYYCASRDYDYDGRYFDYWGRGTLVTVSSASTKGPSVFPLAPCSKSTSGGTAALGCLVKDYFPEPVTVSWNSGALTSGVHTFPAVLQSSGLYSLSSVVTVPSSSLGTQTYICNVNHKPSNTKVDKKVEPDSGDKTHTCPPCPAPELLGGPSVFLFPPKPKDTLMISRTPEVTCVVVDVSHEDPEVKFNWYVDGVEVHNAKTKPREEQYNSTYRVVSVLTVLHQDWLNGKEYKCKVSNKALPAPIEKTISKAKGQPREPQVYTLPPSREEMTKNQVSLVCLVKGFYPSDIAVEWESNGQPENNYKTTPPVLDSDGSFFLYSVLTVDKSRWQQGNVFSCSVMHEALHNHYTQKSLSLSPGK

SEQ ID NO: 31 - protein, 451 aa, Artificial Sequence
  Synthetic Construct
QVQLVQSGAEVKKPGASVKVSCKASGYTFTSHWMHWVRYAPGQGLEWIGEFNPSNGRTNYNEKFKSKATMTVDTSTNTAYMELSSLRSEDTAVYYCASRDYDYDGRYFDYWGRGTLVTVSSASTKGPSVFPLAPCSKSTSGGTAALGCLVKDYFPEPVTVSWNSGALTSGVHTFPAVLQSSGLYSLSSVVTVPSSSLGTQTYICNVNHKPSNTKVDKKVEPDSGDKTHTCPPCPAPELLGGPSVFLFPPKPKDTLMISRTPEVTCVVVDVSHEDPEVKFNWYVDGVEVHNAKTKPREEQYNSTYRVVSVLTVLHQDWLNGKEYKCKVSNKALPAPIEKTISKAKGQPREPQVYTLPPSREEMTDNQVSLTCLVKGFYPSDIAVEWESNGQPENNYKTTPPVLMSDGSFFLASKLTVDKSRWQQGNVFSCSVMHEALHNHYTQKSLSLSPGK

SEQ ID NO: 32 - protein, 451 aa, Artificial Sequence
  Synthetic Construct
QVQLVQSGAEVKKPGASVKVSCKASGYTFTSHWMHWVRYAPGQGLEWIGEFNPSNGRTNYNEKFKSKATMTVDTSTNTAYMELSSLRSEDTAVYYCASRDYDYDGRYFDYWGRGTLVTVSSASTKGPSVFPLAPCSKSTSGGTAALGCLVKDYFPEPVTVSWNSGALTSGVHTFPAVLQSSGLYSLSSVVTVPSSSLGTQTYICNVNHKPSNTKVDKKVEPDSGDKTHTCPPCPAPELLGGPSVFLFPPKPKDTLMISRTPEVTCVVVDVSHEDPEVKFNWYVDGVEVHNAKTKPREEQYNSTYRVVSVLTVLHQDWLNGKEYKCKVSNKALPAPIEKTISKAKGQPRRPRVYTLPPSREEMTKNQVSLVCLVKGFYPSDIAVEWESNGQPENNYKTTPPVLDSDGSFFLYSVLTVDKSRWQQGNVFSCSVMHEALHNHYTQKSLSLSPGK

SEQ ID NO: 33 - protein, 451 aa, Artificial Sequence
  Synthetic Construct
QVQLVQSGAEVKKPGASVKVSCKASGYTFTSHWMHWVRYAPGQGLEWIGEFNPSNGRTNYNEKFKSKATMTVDTSTNTAYMELSSLRSEDTAVYYCASRDYDYDGRYFDYWGRGTLVTVSSASTKGPSVFPLAPCSKSTSGGTAALGCLVKDYFPEPVTVSWNSGALTSGVHTFPAVLQSSGLYSLSSVVTVPSSSLGTQTYICNVNHKPSNTKVDKKVEPDSGDKTHTCPPCPAPELLGGPSVFLFPPKPKDTLMISRTPEVTCVVVDVSHEDPEVKFNWYVDGVEVHNAKTKPREEQYNSTYRVVSVLTVLHQDWLNGKEYKCKVSNKALPAPIEKTISKAKGQPREPQVYTLPPSREDMTKNQVQLTCLVKGFYPSDIAVEWESNGQPENNYKTTPPVLDSDGSFFLASKLTVDKSRWQQGNVFSCSVMHEALHNHYTQKSLSLSPGK

SEQ ID NO: 34 - protein, 451 aa, Artificial Sequence
  Synthetic Construct
QVQLVQSGAEVKKPGASVKVSCKASGYTFTSHWMHWVRYAPGQGLEWIGEFNPSNGRTNYNEKFKSKATMTVDTSTNTAYMELSSLRSEDTAVYYCASRDYDYDGRYFDYWGRGTLVTVSSASTKGPSVFPLAPCSKSTSGGTAALGCLVKDYFPEPVTVSWNSGALTSGVHTFPAVLQSSGLYSLSSVVTVPSSSLGTQTYICNVNHKPSNTKVDKKVEPDSGDKTHTCPPCPAPELLGGPSVFLFPPKPKDTLMISRTPEVTCVVVDVSHEDPEVKFNWYVDGVEVHNAKTKPREEQYNSTYRVVSVLTVLHQDWLNGKEYKCKVSNKALPAPIEKTISKAKGQPREPQVYTLPPSRGDMTKNQVQLTCLVKGFYPSDIAVEWESNGQPENNYKTTPPVLDSDGSFFLASKLTVDKSRWQQGNVFSCSVMHEALHNHYTQKSLSLSPGK

SEQ ID NO: 35 - protein, 451 aa, Artificial Sequence
  Synthetic Construct
QVQLVQSGAEVKKPGASVKVSCKASGYTFTSHWMHWVRYAPGQGLEWIGEFNPSNGRTNYNEKFKSKATMTVDTSTNTAYMELSSLRSEDTAVYYCASRDYDYDGRYFDYWGRGTLVTVSSASTKGPSVFPLAPCSKSTSGGTAALGCLVKDYFPEPVTVSWNSGALTSGVHTFPAVLQSSGLYSLSSVVTVPSSSLGTQTYICNVNHKPSNTKVDKKVEPDSGDKTHTCPPCPAPELLGGPSVFLFPPKPKDTLMISRTPEVTCVVVDVSHEDPEVKFNWYVDGVEVHNAKTKPREEQYNSTYRVVSVLTVLHQDWLNGKEYKCKVSNKALPAPIEKTISKAKGQPREPQVYTLPPSREDMTKNQVRLTCLVKGFYPSDIAVEWESNGQPENNYKTTPPVLDSDGSFFLASKLTVDKSRWQQGNVFSCSVMHEALHNHYTQKSLSLSPGK

SEQ ID NO: 36 - protein, 213 aa, Artificial Sequence
  Synthetic Construct
DIQMTQSPSSLSASVGDRVTITCSASSSVTYMYWYQRKPGDAPKLLIYDTSNLASGVPSRFSGSGSGTDYTFTISSLQPEDIATYYCQQWSSHIFTFGQGTKVEIKRTVAAPSVFIFPPSKEQLKSGTASVVCLLNNFYPREAKVQWKVDNALQSGNSQESVTEQDSKDSTYSLSSTLTLSKADYEKHKVYACEVTHQGLSSPVTKSFNRGEC

SEQ ID NO: 37 - protein, 217 aa, Artificial Sequence
  Synthetic Construct
APELLGGPSVFLFPPKPKDTLMISRTPEVTCVVVDVSHEDPEVKFNWYVDGVEVHNAKTKPREEQYNSTYRVVSVLTVLHQDWLNGKEYKCKVSNKALPAPIEKTISKAKGQPREPQVYTLPPSREEMTKNQVSLTCLVKGFYPSDIAVEWESNGQPENNYKTTPPVLDSDGSFFLYSKLTVDKSRWQQGNVFSCSVMHEALHNHYTQKSLSLSPGK

SEQ ID NO: 38 - protein, 217 aa, Artificial Sequence
  Synthetic Construct
APELLGGPSVFLFPPKPKDTLMISRTPEVTCVVVDVSHEDPEVKFNWYVDGVEVHNAKTKPREEQYNSTYRVVSVLTVLHQDWLNGKEYKCKVSNKALPAPIEKTISKAKGQPREPQVYTLPPSREEMTKNQVSLTCLVKGFYPSDIAVEWESNGQPENNYKTTPPVLMSDGSFFLASKLTVDKSRWQQGNVFSCSVMHEALHNHYTQKSLSLSPGK

SEQ ID NO: 39 - protein, 217 aa, Artificial Sequence
  Synthetic Construct
APELLGGPSVFLFPPKPKDTLMISRTPEVTCVVVDVSHEDPEVKFNWYVDGVEVHNAKTKPREEQYNSTYRVVSVLTVLHQDWLNGKEYKCKVSNKALPAPIEKTISKAKGQPREPQVYTLPPSREEMTDNQVSLTCLVKGFYPSDIAVEWESNGQPENNYKTTPPVLMSDGSFFLASKLTVDKSRWQQGNVFSCSVMHEALHNHYTQKSLSLSPGK

SEQ ID NO: 40 - protein, 217 aa, Artificial Sequence
  Synthetic Construct
APELLGGPSVFLFPPKPKDTLMISRTPEVTCVVVDVSHEDPEVKFNWYVDGVEVHNAKTKPREEQYNSTYRVVSVLTVLHQDWLNGKEYKCKVSNKALPAPIEKTISKAKGQPREPQVSTLPPSREEMTKNQVSLVCLVYGFYPSDIAVEWESNGQPENNYKTTPPVLDSDGSFFLYSVLTVDKSRWQQGNVFSCSVMHEALHNHYTQKSLSLSPGK

SEQ ID NO: 41 - protein, 217 aa, Artificial Sequence
  Synthetic Construct
APELLGGPSVFLFPPKPKDTLMISRTPEVTCVVVDVSHEDPEVKFNWYVDGVEVHNAKTKPREEQYNSTYRVVSVLTVLHQDWLNGKEYKCKVSNKALPAPIEKTISKAKGQPREPQVSTLPPSREEMTKNQVSLMCLVYGFYPSDIAVEWESNGQPENNYKTTPPVLDSDGSFFLYSVLTVDKSRWQQGNVFSCSVMHEALHNHYTQKSLSLSPGK

SEQ ID NO: 42 - protein, 217 aa, Artificial Sequence
  Synthetic Construct
APELLGGPSVFLFPPKPKDTLMISRTPEVTCVVVDVSHEDPEVKFNWYVDGVEVHNAKTKPREEQYNSTYRVVSVLTVLHQDWLNGKEYKCKVSNKALPAPIEKTISKAKGQPREPQVYTLPPSREEMTKNQVSLVCLVKGFYPSDIAVEWESNGQPENNYKTTPPVLDSDGSFFLYSVLTVDKSRWQQGNVFSCSVMHEALHNHYTQKSLSLSPGK

SEQ ID NO: 43 - protein, 217 aa, Artificial Sequence
  Synthetic Construct
APELLGGPSVFLFPPKPKDTLMISRTPEVTCVVVDVSHEDPEVKFNWYVDGVEVHNAKTKPREEQYNSTYRVVSVLTVLHQDWLNGKEYKCKVSNKALPAPIEKTISKAKGQPRRPRVYTLPPSREEMTKNQVSLVCLVKGFYPSDIAVEWESNGQPENNYKTTPPVLDSDGSFFLYSVLTVDKSRWQQGNVFSCSVMHEALHNHYTQKSLSLSPGK

SEQ ID NO: 44 - protein, 217 aa, Artificial Sequence
  Synthetic Construct
APELLGGPSVFLFPPKPKDTLMISRTPEVTCVVVDVSHEDPEVKFNWYVDGVEVHNAKTKPREEQYNSTYRVVSVLTVLHQDWLNGKEYKCKVSNKALPAPIEKTISKAKGQPREPQVYTLPPSREDMTKNQVQLTCLVKGFYPSDIAVEWESNGQPENNYKTTPPVLDSDGSFFLASKLTVDKSRWQQGNVFSCSVMHEALHNHYTQKSLSLSPGK

SEQ ID NO: 45 - protein, 217 aa, Artificial Sequence
  Synthetic Construct
APELLGGPSVFLFPPKPKDTLMISRTPEVTCVVVDVSHEDPEVKFNWYVDGVEVHNAKTKPREEQYNSTYRVVSVLTVLHQDWLNGKEYKCKVSNKALPAPIEKTISKAKGQPREPQVYTLPPSRGDMTKNQVQLTCLVKGFYPSDIAVEWESNGQPENNYKTTPPVLDSDGSFFLASKLTVDKSRWQQGNVFSCSVMHEALHNHYTQKSLSLSPGK

SEQ ID NO: 46 - protein, 217 aa, Artificial Sequence
  Synthetic Construct
APELLGGPSVFLFPPKPKDTLMISRTPEVTCVVVDVSHEDPEVKFNWYVDGVEVHNAKTKPREEQYNSTYRVVSVLTVLHQDWLNGKEYKCKVSNKALPAPIEKTISKAKGQPREPQVYTLPPSREDMTKNQVRLTCLVKGFYPSDIAVEWESNGQPENNYKTTPPVLDSDGSFFLASKLTVDKSRWQQGNVFSCSVMHEALHNHYTQKSLSLSPGK

SEQ ID NO: 47 - protein, 445 aa, Artificial Sequence
  Synthetic Construct
EVQLVESGGGLVQPGGSLRLSCAASGFTFTDYTMDWVRKAPGKGLEWVADVNPNSGGSIYNQEFKGRFTLSVDRSKNTLYLQMNSLRAEDTAVYYCARNLGPSFYFDYWGQGTLVTVSSASTKGPSVFPLAPCSRSTSESTAALGCLVKDYFPEPVTVSWNSGALTSGVATGPAVLQSSGLYSLSSVVTVPSSSLGTKTYTCNVDHKPSNTKVDKRVESKYGPPCPPCPAPEAAGGPSVFLFPPKPKDTLMISRTPEVTCVVVDVSQEDPEVQFNWYVDGVEVHNAKTKPREEQFQSTYRVVSVLTVLHQDWLNGKEYKCKVSNKGLPSSIEKTISKAKGQPREPQVYTLPPSQEEMTDNQVSLTCLVKGFYPSDIAVEWESNGQPENNYKTTPPVLMSDGSFFLASRLTVDKSRWQEGNVFSCSVMHEALHNHYTQKSLSLSLG

SEQ ID NO: 48 - protein, 445 aa, Artificial Sequence
  Synthetic Construct
EVQLVESGGGLVQPGGSLRLSCAASGFTFTDYTMDWVRKAPGKGLEWVADVNPNSGGSIYNQEFKGRFTLSVDRSKNTLYLQMNSLRAEDTAVYYCARNLGPSFYFDYWGQGTLVTVSSASTKGPSVFPLAPCSRSTSESTAALGCLVKDYFPEPVTVSWNSGALTSGVATGPAVLQSSGLYSLSSVVTVPSSSLGTKTYTCNVDHKPSNTKVDKRVESKYGPPCPPCPAPEAAGGPSVFLFPPKPKDTLMISRTPEVTCVVVDVSQEDPEVQFNWYVDGVEVHNAKTKPREEQFQSTYRVVSVLTVLHQDWLNGKEYKCKVSNKGLPSSIEKTISKAKGQPREPQVSTLPPSQEEMTKNQVSLMCLVYGFYPSDIAVEWESNGQPENNYKTTPPVLDSDGSFFLYSVLTVDKSRWQEGNVFSCSVMHEALHNHYTQKSLSLSLG

SEQ ID NO: 49 - protein, 212 aa, Artificial Sequence; identical to SEQ ID NO: 14
  Synthetic Construct

SEQ ID NO: 50 - protein, 445 aa, Artificial Sequence
  Synthetic Construct
EVQLVESGGGLVQPGGSLRLSCAASGYTFTSYWLHWVRKAPGKGLEWVGMIDPSNSDTRFNPEFKDRFTISADTSKNTAYLQMNSLRAEDTAVYYCATYRSYVTPLDYWGQGTLVTVSSASTKGPSVFPLAPCSRSTSESTAALGCLVKDYFPEPVTVSWNSGALTSGVATGPAVLQSSGLYSLSSVVTVPSSSLGTKTYTCNVDHKPSNTKVDKRVESKYGPPCPPCPAPEAAGGPSVFLFPPKPKDTLMISRTPEVTCVVVDVSQEDPEVQFNWYVDGVEVHNAKTKPREEQFQSTYRVVSVLTVLHQDWLNGKEYKCKVSNKGLPSSIEKTISKAKGQPREPQVYTLPPSQEEMTDNQVSLTCLVKGFYPSDIAVEWESNGQPENNYKTTPPVLMSDGSFFLASRLTVDKSRWQEGNVFSCSVMHEALHNHYTQKSLSLSLG

SEQ ID NO: 51 - protein, 445 aa, Artificial Sequence
  Synthetic Construct
EVQLVESGGGLVQPGGSLRLSCAASGYTFTSYWLHWVRKAPGKGLEWVGMIDPSNSDTRFNPEFKDRFTISADTSKNTAYLQMNSLRAEDTAVYYCATYRSYVTPLDYWGQGTLVTVSSASTKGPSVFPLAPCSRSTSESTAALGCLVKDYFPEPVTVSWNSGALTSGVATGPAVLQSSGLYSLSSVVTVPSSSLGTKTYTCNVDHKPSNTKVDKRVESKYGPPCPPCPAPEAAGGPSVFLFPPKPKDTLMISRTPEVTCVVVDVSQEDPEVQFNWYVDGVEVHNAKTKPREEQFQSTYRVVSVLTVLHQDWLNGKEYKCKVSNKGLPSSIEKTISKAKGQPREPQVSTLPPSQEEMTKNQVSLMCLVYGFYPSDIAVEWESNGQPENNYKTTPPVLDSDGSFFLYSVLTVDKSRWQEGNVFSCSVMHEALHNHYTQKSLSLSLG

SEQ ID NO: 52 - protein, 218 aa, Artificial Sequence; identical to SEQ ID NO: 20
  Synthetic Construct

SEQ ID NO: 53 - protein, 447 aa, Artificial Sequence
  Synthetic Construct
QVQLVQSGAEVKKPGASVKVSCKASGYTFTSHWMHWVRYAPGQGLEWIGEFNPSNGRTNYNEKFKSKATMTVDTSTNTAYMELSSLRSEDTAVYYCASRDYDYDGRYFDYWGRGTLVTVSSASTKGPSVFPLAPCSRSTSESTAALGCLVKDYFPEPVTVSWNSGALTSGVHTFPAVLQSSGLYSLSSVVTVPSSSLGTKTYTCNVDHKPSNTKVDKRVESDYGPPCPPCPAPEAAGGPSVFLFPPKPKDTLMISRTPEVTCVVVDVSQEDPEVQFNWYVDGVEVHNAKTKPREEQFQSTYRVVSVLTVLHQDWLNGKEYKCKVSNKGLPSSIEKTISKAKGQPRRPRVYTLPPSQEEMTKNQVSLVCLVKGFYPSDIAVEWESNGQPENNYKTTPPVLDSDGSFFLYSVLTVDKSRWQEGNVFSCSVMHEALHNHYTQKSLSLSLG

SEQ ID NO: 54 - protein, 447 aa, Artificial Sequence
  Synthetic Construct
QVQLVQSGAEVKKPGASVKVSCKASGYTFTSHWMHWVRYAPGQGLEWIGEFNPSNGRTNYNEKFKSKATMTVDTSTNTAYMELSSLRSEDTAVYYCASRDYDYDGRYFDYWGRGTLVTVSSASTKGPSVFPLAPCSRSTSESTAALGCLVKDYFPEPVTVSWNSGALTSGVHTFPAVLQSSGLYSLSSVVTVPSSSLGTKTYTCNVDHKPSNTKVDKRVESDYGPPCPPCPAPEAAGGPSVFLFPPKPKDTLMISRTPEVTCVVVDVSQEDPEVQFNWYVDGVEVHNAKTKPREEQFQSTYRVVSVLTVLHQDWLNGKEYKCKVSNKGLPSSIEKTISKAKGQPREPQVYTLPPSQGDMTKNQVQLTCLVKGFYPSDIAVEWESNGQPENNYKTTPPVLDSDGSFFLASRLTVDKSRWQEGNVFSCSVMHEALHNHYTQKSLSLSLG

SEQ ID NO: 55 - protein, 213 aa, Artificial Sequence; identical to SEQ ID NO: 36
  Synthetic Construct

SEQ ID NO: 56 - protein, 442 aa, Artificial Sequence
  Synthetic Construct
QVQLVQSGAEVKKPGSSVKVSCKASGYTFTTYYLHWVRYAPGQGLEWMGWIYPGNVHAQYNEKFKGRVTITADKSTSTAYMELSSLRSEDTAVYYCARSWEGFPYWGRGTTVTVSSASTKGPSVFPLAPCSRSTSESTAALGCLVKDYFPEPVTVSWNSGALTSGVHTFPAVLQSSGLYSLSSVVTVPSSSLGTKTYTCNVDHKPSNTKVDKRVESDYGPPCPPCPAPEAAGGPSVFLFPPKPKDTLMISRTPEVTCVVVDVSQEDPEVQFNWYVDGVEVHNAKTKPREEQFQSTYRVVSVLTVLHQDWLNGKEYKCKVSNKGLPSSIEKTISKAKGQPRRPRVYTLPPSQEEMTKNQVSLVCLVKGFYPSDIAVEWESNGQPENNYKTTPPVLDSDGSFFLYSVLTVDKSRWQEGNVFSCSVMHEALHNHYTQKSLSLSLG

SEQ ID NO: 57 - protein, 442 aa, Artificial Sequence
  Synthetic Construct
QVQLVQSGAEVKKPGSSVKVSCKASGYTFTTYYLHWVRYAPGQGLEWMGWIYPGNVHAQYNEKFKGRVTITADKSTSTAYMELSSLRSEDTAVYYCARSWEGFPYWGRGTTVTVSSASTKGPSVFPLAPCSRSTSESTAALGCLVKDYFPEPVTVSWNSGALTSGVHTFPAVLQSSGLYSLSSVVTVPSSSLGTKTYTCNVDHKPSNTKVDKRVESDYGPPCPPCPAPEAAGGPSVFLFPPKPKDTLMISRTPEVTCVVVDVSQEDPEVQFNWYVDGVEVHNAKTKPREEQFQSTYRVVSVLTVLHQDWLNGKEYKCKVSNKGLPSSIEKTISKAKGQPREPQVYTLPPSQGDMTKNQVQLTCLVKGFYPSDIAVEWESNGQPENNYKTTPPVLDSDGSFFLASRLTVDKSRWQEGNVFSCSVMHEALHNHYTQKSLSLSLG

SEQ ID NO: 58 - protein, 214 aa, Artificial Sequence; identical to SEQ ID NO: 27
  Synthetic Construct

SEQ ID NO: 59 - protein, 217 aa, Artificial Sequence
  Synthetic Construct
APEFLGGPSVFLFPPKPKDTLMISRTPEVTCVVVDVSQEDPEVQFNWYVDGVEVHNAKTKPREEQFNSTYRVVSVLTVLHQDWLNGKEYKCKVSNKGLPSSIEKTISKAKGQPREPQVYTLPPSQEEMTKNQVSLTCLVKGFYPSDIAVEWESNGQPENNYKTTPPVLDSDGSFFLYSRLTVDKSRWQEGNVFSCSVMHEALHNHYTQKSLSLSLGK

SEQ ID NO: 60 - protein, 217 aa, Artificial Sequence
  Synthetic Construct
APEFLGGPSVFLFPPKPKDTLMISRTPEVTCVVVDVSQEDPEVQFNWYVDGVEVHNAKTKPREEQFNSTYRVVSVLTVLHQDWLNGKEYKCKVSNKGLPSSIEKTISKAKGQPREPQVYTLPPSQEEMTKNQVSLTCLVKGFYPSDIAVEWESNGQPENNYKTTPPVLDSDGSFFLASRLTVDKSRWQEGNVFSCSVMHEALHNHYTQKSLSLSLGK

SEQ ID NO: 61 - protein, 217 aa, Artificial Sequence
  Synthetic Construct
APEFLGGPSVFLFPPKPKDTLMISRTPEVTCVVVDVSQEDPEVQFNWYVDGVEVHNAKTKPREEQFNSTYRVVSVLTVLHQDWLNGKEYKCKVSNKGLPSSIEKTISKAKGQPREPQVYTLPPSQEEMTKNQVSLTCLVKGFYPSDIAVEWESNGQPENNYKTTPPVLMSDGSFFLASRLTVDKSRWQEGNVFSCSVMHEALHNHYTQKSLSLSLGK

SEQ ID NO: 62 - protein, 217 aa, Artificial Sequence
  Synthetic Construct
APEFLGGPSVFLFPPKPKDTLMISRTPEVTCVVVDVSQEDPEVQFNWYVDGVEVHNAKTKPREEQFNSTYRVVSVLTVLHQDWLNGKEYKCKVSNKGLPSSIEKTISKAKGQPREPQVYTLPPSQEEMTDNQVSLTCLVKGFYPSDIAVEWESNGQPENNYKTTPPVLMSDGSFFLASRLTVDKSRWQEGNVFSCSVMHEALHNHYTQKSLSLSLGK

SEQ ID NO: 63 - protein, 217 aa, Artificial Sequence
  Synthetic Construct
APEFLGGPSVFLFPPKPKDTLMISRTPEVTCVVVDVSQEDPEVQFNWYVDGVEVHNAKTKPREEQFNSTYRVVSVLTVLHQDWLNGKEYKCKVSNKGLPSSIEKTISKAKGQPREPQVSTLPPSQEEMTKNQVSLVCLVYGFYPSDIAVEWESNGQPENNYKTTPPVLDSDGSFFLYSVLTVDKSRWQEGNVFSCSVMHEALHNHYTQKSLSLSLGK

SEQ ID NO: 64 - protein, 217 aa, Artificial Sequence
  Synthetic Construct
APEFLGGPSVFLFPPKPKDTLMISRTPEVTCVVVDVSQEDPEVQFNWYVDGVEVHNAKTKPREEQFNSTYRVVSVLTVLHQDWLNGKEYKCKVSNKGLPSSIEKTISKAKGQPREPQVSTLPPSQEEMTKNQVSLMCLVYGFYPSDIAVEWESNGQPENNYKTTPPVLDSDGSFFLYSVLTVDKSRWQEGNVFSCSVMHEALHNHYTQKSLSLSLGK

SEQ ID NO: 65 - protein, 217 aa, Artificial Sequence
  Synthetic Construct
APEFLGGPSVFLFPPKPKDTLMISRTPEVTCVVVDVSQEDPEVQFNWYVDGVEVHNAKTKPREEQFNSTYRVVSVLTVLHQDWLNGKEYKCKVSNKGLPSSIEKTISKAKGQPREPQVYTLPPSQEEMTKNQVSLVCLVKGFYPSDIAVEWESNGQPENNYKTTPPVLDSDGSFFLYSVLTVDKSRWQEGNVFSCSVMHEALHNHYTQKSLSLSLGK

SEQ ID NO: 66 - protein, 217 aa, Artificial Sequence
  Synthetic Construct
APEFLGGPSVFLFPPKPKDTLMISRTPEVTCVVVDVSQEDPEVQFNWYVDGVEVHNAKTKPREEQFNSTYRVVSVLTVLHQDWLNGKEYKCKVSNKGLPSSIEKTISKAKGQPRRPRVYTLPPSQEEMTKNQVSLVCLVKGFYPSDIAVEWESNGQPENNYKTTPPVLDSDGSFFLYSVLTVDKSRWQEGNVFSCSVMHEALHNHYTQKSLSLSLGK

SEQ ID NO: 67 - protein, 217 aa, Artificial Sequence
  Synthetic Construct
APEFLGGPSVFLFPPKPKDTLMISRTPEVTCVVVDVSQEDPEVQFNWYVDGVEVHNAKTKPREEQFNSTYRVVSVLTVLHQDWLNGKEYKCKVSNKGLPSSIEKTISKAKGQPREPQVYTLPPSQEDMTKNQVQLTCLVKGFYPSDIAVEWESNGQPENNYKTTPPVLDSDGSFFLASRLTVDKSRWQEGNVFSCSVMHEALHNHYTQKSLSLSLGK

SEQ ID NO: 68 - protein, 217 aa, Artificial Sequence
  Synthetic Construct
APEFLGGPSVFLFPPKPKDTLMISRTPEVTCVVVDVSQEDPEVQFNWYVDGVEVHNAKTKPREEQFNSTYRVVSVLTVLHQDWLNGKEYKCKVSNKGLPSSIEKTISKAKGQPREPQVYTLPPSQGDMTKNQVQLTCLVKGFYPSDIAVEWESNGQPENNYKTTPPVLDSDGSFFLASRLTVDKSRWQEGNVFSCSVMHEALHNHYTQKSLSLSLGK

SEQ ID NO: 69 - protein, 217 aa, Artificial Sequence
  Synthetic Construct
APEFLGGPSVFLFPPKPKDTLMISRTPEVTCVVVDVSQEDPEVQFNWYVDGVEVHNAKTKPREEQFNSTYRVVSVLTVLHQDWLNGKEYKCKVSNKGLPSSIEKTISKAKGQPREPQVYTLPPSQEDMTKNQVRLTCLVKGFYPSDIAVEWESNGQPENNYKTTPPVLDSDGSFFLASRLTVDKSRWQEGNVFSCSVMHEALHNHYTQKSLSLSLGK